European Patent Specification EP 4 514 846 B1, published September 16, 2026. Title: MULTISPECIFIC ANTIBODIES TARGETING IL-13 and IL-18. Applicant: Novartis AG. Application WO. The sequence listing filed with the application follows.

SEQUENCE LISTING (91 sequences)

SEQ ID NO: 1 - protein, 13 aa, synthetic construct
  REGION 1..13: note = Synthetic polypeptide
SGSSSNIGNHYVN

SEQ ID NO: 2 - protein, 7 aa, synthetic construct
  REGION 1..7: note = Synthetic polypeptide
RNNHRPS

SEQ ID NO: 3 - protein, 11 aa, synthetic construct
  REGION 1..11: note = Synthetic polypeptide
QSWDYSGFSTV

SEQ ID NO: 4 - protein, 13 aa, synthetic construct
  REGION 1..13: note = Synthetic polypeptide
SGSSSNIGNHYVN

SEQ ID NO: 5 - protein, 7 aa, synthetic construct
  REGION 1..7: note = Synthetic polypeptide
RNNHRPS

SEQ ID NO: 6 - protein, 11 aa, synthetic construct
  REGION 1..11: note = Synthetic polypeptide
QSWDYSGFSTV

SEQ ID NO: 7 - protein, 9 aa, synthetic construct
  REGION 1..9: note = Synthetic polypeptide
SSSNIGNHY

SEQ ID NO: 8 - skipped

SEQ ID NO: 9 - protein, 8 aa, synthetic construct
  REGION 1..8: note = Synthetic polypeptide
WDYSGFST

SEQ ID NO: 10 - protein, 8 aa, synthetic construct
  REGION 1..8: note = Synthetic polypeptide
SSNIGNHY

SEQ ID NO: 11 - skipped

SEQ ID NO: 12 - protein, 11 aa, synthetic construct
  REGION 1..11: note = Synthetic polypeptide
QSWDYSGFSTV

SEQ ID NO: 13 - protein, 110 aa, synthetic construct
  REGION 1..110: note = Synthetic polypeptide
DIVLTQPPSVSGAPGQRVTISCSGSSSNIGNHYVNWYQQLPGTAPKLLIYRNNHRPSGVPDRFSGSKSGTSASLAITGLQSEDEADYYCQSWDYSGFSTVFGGGTKLTVL

SEQ ID NO: 14 - protein, 216 aa, synthetic construct
  REGION 1..216: note = Synthetic polypeptide
DIVLTQPPSVSGAPGQRVTISCSGSSSNIGNHYVNWYQQLPGTAPKLLIYRNNHRPSGVPDRFSGSKSGTSASLAITGLQSEDEADYYCQSWDYSGFSTVFGGGTKLTVLGQPKAAPSVTLFPPSSEELQANKATLVCLISDFYPGAVTVAWKADSSPVKAGVETTTPSKQSNNKYAASSYLSLTPEQWKSHRSYSCQVTHEGSTVEKTVAPTECS

SEQ ID NO: 15 - protein, 15 aa, synthetic construct
  REGION 1..15: note = Synthetic polypeptide
RASKSVDSYGNSFMH

SEQ ID NO: 16 - protein, 7 aa, synthetic construct
  REGION 1..7: note = Synthetic polypeptide
LASNLES

SEQ ID NO: 17 - protein, 9 aa, synthetic construct
  REGION 1..9: note = Synthetic polypeptide
QQNNEDPRT

SEQ ID NO: 18 - protein, 15 aa, synthetic construct
  REGION 1..15: note = Synthetic polypeptide
RASKSVDSYGNSFMH

SEQ ID NO: 19 - protein, 7 aa, synthetic construct
  REGION 1..7: note = Synthetic polypeptide
LASNLES

SEQ ID NO: 20 - protein, 9 aa, synthetic construct
  REGION 1..9: note = Synthetic polypeptide
QQNNEDPRT

SEQ ID NO: 21 - protein, 11 aa, synthetic construct
  REGION 1..11: note = Synthetic polypeptide
SKSVDSYGNSF

SEQ ID NO: 22 - skipped

SEQ ID NO: 23 - protein, 6 aa, synthetic construct
  REGION 1..6: note = Synthetic polypeptide
NNEDPR

SEQ ID NO: 24 - protein, 10 aa, synthetic construct
  REGION 1..10: note = Synthetic polypeptide
KSVDSYGNSF

SEQ ID NO: 25 - skipped

SEQ ID NO: 26 - protein, 9 aa, synthetic construct
  REGION 1..9: note = Synthetic polypeptide
QQNNEDPRT

SEQ ID NO: 27 - protein, 111 aa, synthetic construct [sequence omitted]

SEQ ID NO: 28 - protein, 218 aa, synthetic construct
  REGION 1..218: note = Synthetic polypeptide
DIVMTQSPDSLSVSLGERATINCRASKSVDSYGNSFMHWYQQKPGQPPKLLIYLASNLESGVPDRFSGSGSGTDFTLTISSLQAEDVAVYYCQQNNEDPRTFGGGTKVEIKRTVAAPSVFIFPPSDEQLKSGTASVVCLLNNFYPREAKVQWKVDNALQSGNSQESVTEQDSKDSTYSLSSTLTLSKADYEKHKVYACEVTHQGLSSPVTKSFNRGEC

SEQ ID NO: 29 - protein, 10 aa, synthetic construct
  REGION 1..10: note = Synthetic polypeptide
GGTFKSYAIS

SEQ ID NO: 30 - protein, 17 aa, synthetic construct
  REGION 1..17: note = Synthetic polypeptide
NIIPMTGQTYYAQKFQG

SEQ ID NO: 31 - protein, 10 aa, synthetic construct
  REGION 1..10: note = Synthetic polypeptide
AAYHPLVFDN

SEQ ID NO: 32 - protein, 5 aa, synthetic construct
  REGION 1..5: note = Synthetic polypeptide
SYAIS

SEQ ID NO: 33 - protein, 17 aa, synthetic construct
  REGION 1..17: note = Synthetic polypeptide
NIIPMTGQTYYAQKFQG

SEQ ID NO: 34 - protein, 10 aa, synthetic construct
  REGION 1..10: note = Synthetic polypeptide
AAYHPLVFDN

SEQ ID NO: 35 - protein, 7 aa, synthetic construct
  REGION 1..7: note = Synthetic polypeptide
GGTFKSY

SEQ ID NO: 36 - protein, 6 aa, synthetic construct
  REGION 1..6: note = Synthetic polypeptide
IPMTGQ

SEQ ID NO: 37 - protein, 10 aa, synthetic construct
  REGION 1..10: note = Synthetic polypeptide
AAYHPLVFDN

SEQ ID NO: 38 - protein, 8 aa, synthetic construct
  REGION 1..8: note = Synthetic polypeptide
GGTFKSYA

SEQ ID NO: 39 - protein, 8 aa, synthetic construct
  REGION 1..8: note = Synthetic polypeptide
IIPMTGQT

SEQ ID NO: 40 - protein, 12 aa, synthetic construct
  REGION 1..12: note = Synthetic polypeptide
ARAAYHPLVFDN

SEQ ID NO: 41 - protein, 119 aa, synthetic construct
  REGION 1..119: note = Synthetic polypeptide
EVQLVQSGAEVKKPGSSVKVSCKASGGTFKSYAISWVRQAPGQGLEWMGNIIPMTGQTYYAQKFQGRVTITADESTSTAYMELSSLRSEDTAVYYCARAAYHPLVFDNWGQGTLVTVSS

SEQ ID NO: 42 - protein, 449 aa, synthetic construct
  REGION 1..449: note = Synthetic polypeptide
EVQLVQSGAEVKKPGSSVKVSCKASGGTFKSYAISWVRQAPGQGLEWMGNIIPMTGQTYYAQKFQGRVTITADESTSTAYMELSSLRSEDTAVYYCARAAYHPLVFDNWGQGTLVTVSSASTKGPSVFPLAPSSKSTSGGTAALGCLVKDYFPEPVTVSWNSGALTSGVHTFPAVLQSSGLYSLSSVVTVPSSSLGTQTYICNVNHKPSNTKVDKRVEPKSCDKTHTCPPCPAPELLGGPSVFLFPPKPKDTLYITREPEVTCVVVDVSHEDPEVKFNWYVDGVEVHNAKTKPREEQYNSTYRVVSVLTVLHQDWLNGKEYKCKVSNKALPAPIEKTISKAKGQPREPQVCTLPPSREEMTKNQVSLSCAVKGFYPSDIAVEWESNGQPENNYKTTPPVLDSDGSFFLVSKLTVDKSRWQQGNVFSCSVMHEALHNHYTQKSLSLSPGK

SEQ ID NO: 43 - protein, 10 aa, synthetic construct
  REGION 1..10: note = Synthetic polypeptide
GFSLSAYSVN

SEQ ID NO: 44 - protein, 16 aa, synthetic construct
  REGION 1..16: note = Synthetic polypeptide
MIWGDGKIVYNSALKS

SEQ ID NO: 45 - protein, 10 aa, synthetic construct
  REGION 1..10: note = Synthetic polypeptide
DGYYPYAMDN

SEQ ID NO: 46 - protein, 5 aa, synthetic construct
  REGION 1..5: note = Synthetic polypeptide
AYSVN

SEQ ID NO: 47 - protein, 16 aa, synthetic construct
  REGION 1..16: note = Synthetic polypeptide
MIWGDGKIVYNSALKS

SEQ ID NO: 48 - protein, 10 aa, synthetic construct
  REGION 1..10: note = Synthetic polypeptide
DGYYPYAMDN

SEQ ID NO: 49 - protein, 7 aa, synthetic construct
  REGION 1..7: note = Synthetic polypeptide
GFSLSAY

SEQ ID NO: 50 - protein, 5 aa, synthetic construct
  REGION 1..5: note = Synthetic polypeptide
WGDGK

SEQ ID NO: 51 - protein, 10 aa, synthetic construct
  REGION 1..10: note = Synthetic polypeptide
DGYYPYAMDN

SEQ ID NO: 52 - protein, 8 aa, synthetic construct
  REGION 1..8: note = Synthetic polypeptide
GFSLSAYS

SEQ ID NO: 53 - protein, 7 aa, synthetic construct
  REGION 1..7: note = Synthetic polypeptide
IWGDGKI

SEQ ID NO: 54 - protein, 12 aa, synthetic construct
  REGION 1..12: note = Synthetic polypeptide
AGDGYYPYAMDN

SEQ ID NO: 55 - protein, 118 aa, synthetic construct [sequence omitted]

SEQ ID NO: 56 - protein, 448 aa, synthetic construct
  REGION 1..448: note = Synthetic polypeptide
QVTLRESGPALVKPTQTLTLTCTVSGFSLSAYSVNWIRQPPGKALEWLAMIWGDGKIVYNSALKSRLTISKDTSKNQVVLTMTNMDPVDTATYYCAGDGYYPYAMDNWGQGSLVTVSSASTKGPSVFPLAPSSKSTSGGTAALGCLVKDYFPEPVTVSWNSGALTSGVHTFPAVLQSSGLYSLSSVVTVPSSSLGTQTYICNVNHKPSNTKVDKRVEPKSCDKTHTCPPCPAPELLGGPSVFLFPPKPKDTLYITREPEVTCVVVDVSHEDPEVKFNWYVDGVEVHNAKTKPREEQYNSTYRVVSVLTVLHQDWLNGKEYKCKVSNKALPAPIEKTISKAKGQPREPQVYTLPPCREEMTKNQVSLWCLVKGFYPSDIAVEWESNGQPENNYKTTPPVLDSDGSFFLYSKLTVDKSRWQQGNVFSCSVMHEALHNHYTQKSLSLSPGK

SEQ ID NO: 57 - protein, 449 aa, synthetic construct
  REGION 1..449: note = Synthetic polypeptide
EVQLVQSGAEVKKPGSSVKVSCKASGGTFKSYAISWVRQAPGQGLEWMGNIIPMTGQTYYAQKFQGRVTITADESTSTAYMELSSLRSEDTAVYYCARAAYHPLVFDNWGQGTLVTVSSASTKGPSVFPLAPSSKSTSGGTAALGCLVKDYFPEPVTVSWNSGALTSGVHTFPAVLQSSGLYSLSSVVTVPSSSLGTQTYICNVNHKPSNTKVDKRVEPKSCDKTHTCPPCPAPELLGGPSVFLFPPKPKDTLYITREPEVTCVVVDVSHEDPEVKFNWYVDGVEVHNAKTKPREEQYNSTYRVVSVLTVLHQDWLNGKEYKCKVSNKALPAPIEKTISKAKGQPREPQVYTLPPCREEMTKNQVSLWCLVKGFYPSDIAVEWESNGQPENNYKTTPPVLDSDGSFFLYSKLTVDKSRWQQGNVFSCSVMHEALHNHYTQKSLSLSPGK

SEQ ID NO: 58 - protein, 448 aa, synthetic construct
  REGION 1..448: note = Synthetic polypeptide
QVTLRESGPALVKPTQTLTLTCTVSGFSLSAYSVNWIRQPPGKALEWLAMIWGDGKIVYNSALKSRLTISKDTSKNQVVLTMTNMDPVDTATYYCAGDGYYPYAMDNWGQGSLVTVSSASTKGPSVFPLAPSSKSTSGGTAALGCLVKDYFPEPVTVSWNSGALTSGVHTFPAVLQSSGLYSLSSVVTVPSSSLGTQTYICNVNHKPSNTKVDKRVEPKSCDKTHTCPPCPAPELLGGPSVFLFPPKPKDTLYITREPEVTCVVVDVSHEDPEVKFNWYVDGVEVHNAKTKPREEQYNSTYRVVSVLTVLHQDWLNGKEYKCKVSNKALPAPIEKTISKAKGQPREPQVCTLPPSREEMTKNQVSLSCAVKGFYPSDIAVEWESNGQPENNYKTTPPVLDSDGSFFLVSKLTVDKSRWQQGNVFSCSVMHEALHNHYTQKSLSLSPGK

SEQ ID NO: 59 - protein, 11 aa, synthetic construct
  REGION 1..11: note = Synthetic polypeptide
RAGQSVSSYLV

SEQ ID NO: 60 - protein, 7 aa, synthetic construct
  REGION 1..7: note = Synthetic polypeptide
DASNRAT

SEQ ID NO: 61 - protein, 11 aa, synthetic construct
  REGION 1..11: note = Synthetic polypeptide
QQRSSWPPVYT

SEQ ID NO: 62 - protein, 11 aa, synthetic construct
  REGION 1..11: note = Synthetic polypeptide
RAGQSVSSYLV

SEQ ID NO: 63 - protein, 7 aa, synthetic construct
  REGION 1..7: note = Synthetic polypeptide
DASNRAT

SEQ ID NO: 64 - protein, 11 aa, synthetic construct
  REGION 1..11: note = Synthetic polypeptide
QQRSSWPPVYT

SEQ ID NO: 65 - protein, 7 aa, synthetic construct
  REGION 1..7: note = Synthetic polypeptide
GQSVSSY

SEQ ID NO: 66 - skipped

SEQ ID NO: 67 - protein, 8 aa, synthetic construct
  REGION 1..8: note = Synthetic polypeptide
RSSWPPVY

SEQ ID NO: 68 - protein, 6 aa, synthetic construct
  REGION 1..6: note = Synthetic polypeptide
QSVSSY

SEQ ID NO: 69 - skipped

SEQ ID NO: 70 - protein, 11 aa, synthetic construct
  REGION 1..11: note = Synthetic polypeptide
QQRSSWPPVYT

SEQ ID NO: 71 - protein, 109 aa, synthetic construct
  REGION 1..109: note = Synthetic polypeptide
EIVLTQSPATLSLSPGERAILSCRAGQSVSSYLVWYQQKPGQAPRLLIYDASNRATGIPARFSGSGSGTDFTLTISSLEPEDFAVYYCQQRSSWPPVYTFGQGTKLEIK

SEQ ID NO: 72 - protein, 216 aa, synthetic construct
  REGION 1..216: note = Synthetic polypeptide
EIVLTQSPATLSLSPGERAILSCRAGQSVSSYLVWYQQKPGQAPRLLIYDASNRATGIPARFSGSGSGTDFTLTISSLEPEDFAVYYCQQRSSWPPVYTFGQGTKLEIKRTVAAPSVFIFPPSDEQLKSGTASVVCLLNNFYPREAKVQWKVDNALQSGNSQESVTEQDSKDSTYSLSSTLTLSKADYEKHKVYACEVTHQGLSSPVTKSFNRGEC

SEQ ID NO: 73 - protein, 10 aa, synthetic construct
  REGION 1..10: note = Synthetic polypeptide
GFTFSSYGMH

SEQ ID NO: 74 - protein, 17 aa, synthetic construct
  REGION 1..17: note = Synthetic polypeptide
IIWYDGSNKYYADSVKG

SEQ ID NO: 75 - protein, 11 aa, synthetic construct
  REGION 1..11: note = Synthetic polypeptide
LWFGDLDAFDI

SEQ ID NO: 76 - protein, 5 aa, synthetic construct
  REGION 1..5: note = Synthetic polypeptide
SYGMH

SEQ ID NO: 77 - protein, 17 aa, synthetic construct
  REGION 1..17: note = Synthetic polypeptide
IIWYDGSNKYYADSVKG

SEQ ID NO: 78 - protein, 11 aa, synthetic construct
  REGION 1..11: note = Synthetic polypeptide
LWFGDLDAFDI

SEQ ID NO: 79 - protein, 7 aa, synthetic construct
  REGION 1..7: note = Synthetic polypeptide
GFTFSSY

SEQ ID NO: 80 - protein, 6 aa, synthetic construct
  REGION 1..6: note = Synthetic polypeptide
WYDGSN

SEQ ID NO: 81 - protein, 11 aa, synthetic construct
  REGION 1..11: note = Synthetic polypeptide
LWFGDLDAFDI

SEQ ID NO: 82 - protein, 8 aa, synthetic construct
  REGION 1..8: note = Synthetic polypeptide
GFTFSSYG

SEQ ID NO: 83 - protein, 8 aa, synthetic construct
  REGION 1..8: note = Synthetic polypeptide
IWYDGSNK

SEQ ID NO: 84 - protein, 13 aa, synthetic construct
  REGION 1..13: note = Synthetic polypeptide
ARLWFGDLDAFDI

SEQ ID NO: 85 - protein, 120 aa, synthetic construct
  REGION 1..120: note = Synthetic polypeptide
EVQLVESGGGVVQPGRSLRLSCAASGFTFSSYGMHWVRQAPGKGLEWVAIIWYDGSNKYYADSVKGRFTISRDNSKNTLYLQMNSLRAEDTAVYYCARLWFGDLDAFDIWGQGTMVTVSS

SEQ ID NO: 86 - protein, 450 aa, synthetic construct
  REGION 1..450: note = Synthetic polypeptide
EVQLVESGGGVVQPGRSLRLSCAASGFTFSSYGMHWVRQAPGKGLEWVAIIWYDGSNKYYADSVKGRFTISRDNSKNTLYLQMNSLRAEDTAVYYCARLWFGDLDAFDIWGQGTMVTVSSASTKGPSVFPLAPSSKSTSGGTAALGCLVKDYFPEPVTVSWNSGALTSGVHTFPAVLQSSGLYSLSSVVTVPSSSLGTQTYICNVNHKPSNTKVDKRVEPKSCDKTHTCPPCPAPELLGGPSVFLFPPKPKDTLYITREPEVTCVVVDVSHEDPEVKFNWYVDGVEVHNAKTKPREEQYNSTYRVVSVLTVLHQDWLNGKEYKCKVSNKALPAPIEKTISKAKGQPREPQVCTLPPSREEMTKNQVSLSCAVKGFYPSDIAVEWESNGQPENNYKTTPPVLDSDGSFFLVSKLTVDKSRWQQGNVFSCSVMHEALHNHYTQKSLSLSPGK

SEQ ID NO: 87 - protein, 449 aa, synthetic construct; identical to SEQ ID NO: 57
  REGION 1..449: note = Synthetic polypeptide

SEQ ID NO: 88 - protein, 449 aa, synthetic construct
  REGION 1..449: note = Synthetic polypeptide
EVQLVQSGAEVKKPGSSVKVSCKASGGTFKSYAISWVRQAPGQGLEWMGNIIPMTGQTYYAQKFQGRVTITADESTSTAYMELSSLRSEDTAVYYCARAAYHPLVFDNWGQGTLVTVSSASTKGPSVFPLAPSSKSTSGGTAALGCLVKDYFPEPVTVSWNSGALTSGVHTFPAVLQSSGLYSLSSVVTVPSSSLGTQTYICNVNHKPSNTKVDKRVEPKSCDKTHTCPPCPAPEAAGGPSVFLFPPKPKDTLYITREPEVTCVVVDVSHEDPEVKFNWYVDGVEVHNAKTKPREEQYNSTYRVVSVLTVLHQDWLNGKEYKCKVSNKALPAPIEKTISKAKGQPREPQVYTLPPCREEMTKNQVSLWCLVKGFYPSDIAVEWESNGQPENNYKTTPPVLDSDGSFFLYSKLTVDKSRWQQGNVFSCSVMHEALHNHYTQKSLSLSPGK

SEQ ID NO: 89 - protein, 448 aa, synthetic construct
  REGION 1..448: note = Synthetic polypeptide
QVTLRESGPALVKPTQTLTLTCTVSGFSLSAYSVNWIRQPPGKALEWLAMIWGDGKIVYNSALKSRLTISKDTSKNQVVLTMTNMDPVDTATYYCAGDGYYPYAMDNWGQGSLVTVSSASTKGPSVFPLAPSSKSTSGGTAALGCLVKDYFPEPVTVSWNSGALTSGVHTFPAVLQSSGLYSLSSVVTVPSSSLGTQTYICNVNHKPSNTKVDKRVEPKSCDKTHTCPPCPAPEAAGGPSVFLFPPKPKDTLYITREPEVTCVVVDVSHEDPEVKFNWYVDGVEVHNAKTKPREEQYNSTYRVVSVLTVLHQDWLNGKEYKCKVSNKALPAPIEKTISKAKGQPREPQVCTLPPSREEMTKNQVSLSCAVKGFYPSDIAVEWESNGQPENNYKTTPPVLDSDGSFFLVSKLTVDKSRWQQGNVFSCSVMHEALHNHYTQKSLSLSPGK

SEQ ID NO: 90 - protein, 449 aa, synthetic construct
  REGION 1..449: note = Synthetic polypeptide
EVQLVQSGAEVKKPGSSVKVSCKASGGTFKSYAISWVRQAPGQGLEWMGNIIPMTGQTYYAQKFQGRVTITADESTSTAYMELSSLRSEDTAVYYCARAAYHPLVFDNWGQGTLVTVSSASTKGPSVFPLAPSSKSTSGGTAALGCLVKDYFPEPVTVSWNSGALTSGVHTFPAVLQSSGLYSLSSVVTVPSSSLGTQTYICNVNHKPSNTKVDKRVEPKSCDKTHTCPPCPAPEAAGGPSVFLFPPKPKDTLYITREPEVTCVVVDVSHEDPEVKFNWYVDGVEVHNAKTKPREEQYNSTYRVVSVLTVLHQDWLNGKEYKCKVSNKALPAPIEKTISKAKGQPREPQVCTLPPSREEMTKNQVSLSCAVKGFYPSDIAVEWESNGQPENNYKTTPPVLDSDGSFFLVSKLTVDKSRWQQGNVFSCSVMHEALHNHYTQKSLSLSPGK

SEQ ID NO: 91 - protein, 448 aa, synthetic construct
  REGION 1..448: note = Synthetic polypeptide
QVTLRESGPALVKPTQTLTLTCTVSGFSLSAYSVNWIRQPPGKALEWLAMIWGDGKIVYNSALKSRLTISKDTSKNQVVLTMTNMDPVDTATYYCAGDGYYPYAMDNWGQGSLVTVSSASTKGPSVFPLAPSSKSTSGGTAALGCLVKDYFPEPVTVSWNSGALTSGVHTFPAVLQSSGLYSLSSVVTVPSSSLGTQTYICNVNHKPSNTKVDKRVEPKSCDKTHTCPPCPAPEAAGGPSVFLFPPKPKDTLYITREPEVTCVVVDVSHEDPEVKFNWYVDGVEVHNAKTKPREEQYNSTYRVVSVLTVLHQDWLNGKEYKCKVSNKALPAPIEKTISKAKGQPREPQVYTLPPCREEMTKNQVSLWCLVKGFYPSDIAVEWESNGQPENNYKTTPPVLDSDGSFFLYSKLTVDKSRWQQGNVFSCSVMHEALHNHYTQKSLSLSPGK